European Patent Specification EP 3 082 848 B1, published October 18, 2023. Title: POPULATION PHARMACOKINETICS TOOLS AND USES THEREOF. Applicant: JIANG, HAIYAN. Application To be assigned. The sequence listing filed with the application follows.

SEQUENCE LISTING (21 sequences)

SEQ ID NO: 1 - DNA, 7583 bp, Artificial Sequence
  pSYN-FIX-030
gcgcgcgttgacattgattattgactagttattaatagtaatcaattacggggtcattagttcatagcccatatatggagttccgcgttacataacttacggtaaatggcccgcctggctgaccgcccaacgacccccgcccattgacgtcaataatgacgtatgttcccatagtaacgccaatagggactttccattgacgtcaatgggtggagtatttacggtaaactgcccacttggcagtacatcaagtgtatcatatgccaagtacgccccctattgacgtcaatgacggtaaatggcccgcctggcattatgcccagtacatgaccttatgggactttcctacttggcagtacatctacgtattagtcatcgctattaccatggtgatgcggttttggcagtacatcaatgggcgtggatagcggtttgactcacggggatttccaagtctccaccccattgacgtcaatgggagtttgttttggcaccaaaatcaacgggactttccaaaatgtcgtaacaactccgccccattgacgcaaatgggcggtaggcgtgtacggtgggaggtctatataagcagagctctctggctaactagagaacccactgcttactggcttatcgaaattaatacgactcactatagggagacccaagcttcgcgacgtacggccgccaccatgcagcgcgtgaacatgatcatggcagaatcaccaggcctcatcaccatctgccttttaggatatctactcagtgctgaatgtacaggtttgtttccttttttaaaatacattgagtatgcttgccttttagatatagaaatatctgatgctgtcttcttcactaaattttgattacatgatttgacagcaatattgaagagtctaacagccagcacgcaggttggtaagtactgtgggaacatcacagattttggctccatgccctaaagagaaattggctttcagattatttggattaaaaacaaagactttcttaagagatgtaaaattttcatgatgttttcttttttgctaaaactaaagaattattcttttacatttcagtttttcttgatcatgaaaacgccaacaaaattctgaatcggccaaagaggtataattcaggtaaattggaagagtttgttcaagggaatctagagagagaatgtatggaagaaaagtgtagttttgaagaagcacgagaagtttttgaaaacactgaaagaacaactgaattttggaagcagtatgttgatggagatcagtgtgagtccaatccatgtttaaatggcggcagttgcaaggatgacattaattcctatgaatgttggtgtccctttggatttgaaggaaagaactgtgaattagatgtaacatgtaacattaagaatggcagatgcgagcagttttgtaaaaatagtgctgataacaaggtggtttgctcctgtactgagggatatcgacttgcagaaaaccagaagtcctgtgaaccagcagtgccatttccatgtggaagagtttctgtttcacaaacttctaagctcacccgtgctgagactgtttttcctgatgtggactatgtaaattctactgaagctgaaaccattttggataacatcactcaaagcacccaatcatttaatgacttcactcgggttgttggtggagaagatgccaaaccaggtcaattcccttggcaggttgttttgaatggtaaagttgatgcattctgtggaggctctatcgttaatgaaaaatggattgtaactgctgcccactgtgttgaaactggtgttaaaattacagttgtcgcaggtgaacataatattgaggagacagaacatacagagcaaaagcgaaatgtgattcgaattattcctcaccacaactacaatgcagctattaataagtacaaccatgacattgcccttctggaactggacgaacccttagtgctaaacagctacgttacacctatttgcattgctgacaaggaatacacgaacatcttcctcaaatttggatctggctatgtaagtggctggggaagagtcttccacaaagggagatcagctttagttcttcagtaccttagagttccacttgttgaccgagccacatgtcttcgatctacaaagttcaccatctataacaacatgttctgtgctggcttccatgaaggaggtagagattcatgtcaaggagatagtgggggaccccatgttactgaagtggaagggaccagtttcttaactggaattattagctggggtgaagagtgtgcaatgaaaggcaaatatggaatatataccaaggtgtcccggtatgtcaactggattaaggaaaaaacaaagctcactgacaaaactcacacatgcccaccgtgcccagctccggaactcctgggcggaccgtcagtcttcctcttccccccaaaacccaaggacaccctcatgatctcccggacccctgaggtcacatgcgtggtggtggacgtgagccacgaagaccctgaggtcaagttcaactggtacgtggacggcgtggaggtgcataatgccaagacaaagccgcgggaggagcagtacaacagcacgtaccgtgtggtcagcgtcctcaccgtcctgcaccaggactggctgaatggcaaggagtacaagtgcaaggtctccaacaaagccctcccagcccccatcgagaaaaccatctccaaagccaaagggcagccccgagaaccacaggtgtacaccctgcccccatcccgggatgagctgaccaagaaccaggtcagcctgacctgcctggtcaaaggcttctatcccagcgacatcgccgtggagtgggagagcaatgggcagccggagaacaactacaagaccacgcctcccgtgttggactccgacggctccttcttcctctacagcaagctcaccgtggacaagagcaggtggcagcaggggaacgtcttctcatgctccgtgatgcatgaggctctgcacaaccactacacgcagaagagcctctccctgtctccgggtaaatgagaattcagacatgataagatacattgatgagtttggacaaaccacaactagaatgcagtgaaaaaaatgctttatttgtgaaatttgtgatgctattgctttatttgtaaccattataagctgcaataaacaagttggggtgggcgaagaactccagcatgagatccccgcgctggaggatcatccagccggcgtcccggaaaacgattccgaagcccaacctttcatagaaggcggcggtggaatcgaaatctcgtagcacgtgtcagtcctgctcctcggccacgaagtgcacgcagttgccggccgggtcgcgcagggcgaactcccgcccccacggctgctcgccgatctcggtcatggccggcccggaggcgtcccggaagttcgtggacacgacctccgaccactcggcgtacagctcgtccaggccgcgcacccacacccaggccagggtgttgtccggcaccacctggtcctggaccgcgctgatgaacagggtcacgtcgtcccggaccacaccggcgaagtcgtcctccacgaagtcccgggagaacccgagccggtcggtccagaactcgaccgctccggcgacgtcgcgcgcggtgagcaccggaacggcactggtcaacttggccatggtttagttcctcaccttgtcgtattatactatgccgatatactatgccgatgattaattgtcaacacgtgctgatcagatccgaaaatggatatacaagctcccgggagctttttgcaaaagcctaggcctccaaaaaagcctcctcactacttctggaatagctcagaggcagaggcggcctcggcctctgcataaataaaaaaaattagtcagccatggggcggagaatgggcggaactgggcggagttaggggcgggatgggcggagttaggggcgggactatggttgctgactaattgagatgcatgctttgcatacttctgcctgctggggagcctggggactttccacacctggttgctgactaattgagatgcatgctttgcatacttctgcctgctggggagcctggggactttccacaccctcgtcgagctagcttcgtgaggctccggtgcccgtcagtgggcagagcgcacatcgcccacagtccccgagaagttggggggaggggtcggcaattgaaccggtgcctagagaaggtggcgcggggtaaactgggaaagtgatgtcgtgtactggctccgcctttttcccgagggtgggggagaaccgtatataagtgcagtagtcgccgtgaacgttctttttcgcaacgggtttgccgccagaacacaggtaagtgccgtgtgtggttcccgcgggcctggcctctttacgggttatggcccttgcgtgccttgaattacttccacctggctccagtacgtgattcttgatcccgagctggagccaggggcgggccttgcgctttaggagccccttcgcctcgtgcttgagttgaggcctggcctgggcgctggggccgccgcgtgcgaatctggtggcaccttcgcgcctgtctcgctgctttcgataagtctctagccatttaaaatttttgatgacctgctgcgacgctttttttctggcaagatagtcttgtaaatgcgggccaggatctgcacactggtatttcggtttttggggccgcgggcggcgacggggcccgtgcgtcccagcgcacatgttcggcgaggcggggcctgcgagcgcggccaccgagaatcggacgggggtagtctcaagctggccggcctgctctggtgcctggcctcgcgccgccgtgtatcgccccgccctgggcggcaaggctggcccggtcggcaccagttgcgtgagcggaaagatggccgcttcccggccctgctccagggggctcaaaatggaggacgcggcgctcgggagagcgggcgggtgagtcacccacacaaaggaaaggggcctttccgtcctcagccgtcgcttcatgtgactccacggagtaccgggcgccgtccaggcacctcgattagttctggagcttttggagtacgtcgtctttaggttggggggaggggttttatgcgatggagtttccccacactgagtgggtggagactgaagttaggccagcttggcacttgatgtaattctccttggaatttgccctttttgagtttggatcttggttcattctcaagcctcagacagtggttcaaagtttttttcttccatttcaggtgtcgtgaacacgtggtcgcggccgcgccgccaccatggagacagacacactcctgctatgggtactgctgctctgggttccaggttccactggtgacaaaactcacacatgcccaccgtgcccagcacctgaactcctgggaggaccgtcagtcttcctcttccccccaaaacccaaggacaccctcatgatctcccggacccctgaggtcacatgcgtggtggtggacgtgagccacgaagaccctgaggtcaagttcaactggtacgtggacggcgtggaggtgcataatgccaagacaaagccgcgggaggagcagtacaacagcacgtaccgtgtggtcagcgtcctcaccgtcctgcaccaggactggctgaatggcaaggagtacaagtgcaaggtctccaacaaagccctcccagcccccatcgagaaaaccatctccaaagccaaagggcagccccgagaaccacaggtgtacaccctgcccccatcccgcgatgagctgaccaagaaccaggtcagcctgacctgcctggtcaaaggcttctatcccagcgacatcgccgtggagtgggagagcaatgggcagccggagaacaactacaagaccacgcctcccgtgttggactccgacggctccttcttcctctacagcaagctcaccgtggacaagagcaggtggcagcaggggaacgtcttctcatgctccgtgatgcatgaggctctgcacaaccactacacgcagaagagcctctccctgtctccgggtaaatgactcgagagatctggccggctgggcccgtttcgaaggtaagcctatccctaaccctctcctcggtctcgattctacgcgtaccggtcatcatcaccatcaccattgagtttaaacccgctgatcagcctcgactgtgccttctagttgccagccatctgttgtttgcccctcccccgtgccttccttgaccctggaaggtgccactcccactgtcctttcctaataaaatgaggaaattgcatcgcattgtctgagtaggtgtcattctattctggggggtggggtggggcaggacagcaagggggaggattgggaagacaatagcaggcatgctggggatgcggtgggctctatggcttctgaggcggaaagaaccagtggcggtaatacggttatccacagaatcaggggataacgcaggaaagaacatgtgagcaaaaggccagcaaaaggccaggaaccgtaaaaaggccgcgttgctggcgtttttccataggctccgcccccctgacgagcatcacaaaaatcgacgctcaagtcagaggtggcgaaacccgacaggactataaagataccaggcgtttccccctagaagctccctcgtgcgctctcctgttccgaccctgccgcttaccggatacctgtccgcctttctcccttcgggaagcgtggcgctttctcatagctcacgctgtaggtatctcagttcggtgtaggtcgttcgctccaagctgggctgtgtgcacgaaccccccgttcagcccgaccgctgcgccttatccggtaactatcgtcttgagtccaacccggtaagacacgacttatcgccactggcagcagccactggtaacaggattagcagagcgaggtatgtaggcggtgctacagagttcttgaagtggtggcctaactacggctacactagaagaacagtatttggtatctgcgctctgctgaagccagttaccttcggaaaaagagttggtagctcttgatccggcaaacaaaccaccgctggtagcggtggtttttttgtttgcaagcagcagattacgcgcagaaaaaaaggatctcaagaagatcctttgatcttttctacggggtctgacgctcagtggaacgaaaactcacgttaagggattttggtcatgacattaacctataaaaataggcgtatcacgaggccctttcgtctcgcgcgtttcggtgatgacggtgaaaacctctgacacatgcagctcccggagacggtcacagcttgtctgtaagcggatgccgggagcagacaagcccgtcagggcgcgtcagcgggtgttggcgggtgtcggggctggcttaactatgcggcatcagagcagattgtactgagagtgcaccatatatgcggtgtgaaataccgcacagatgcgtaaggagaaaataccgcatcaggcgccattcgccattcaggctgcgcaactgttgggaagggcgatcggtgcgggcctcttcgctattacgcca

SEQ ID NO: 2 - protein, 688 aa, Artificial Sequence
  pSYN-FIX-030
  SIGNAL (-46)..(-19)220>
  SIGNAL (-18)..(-1)
  mat_peptide (1)..(642)
MQRVNMIMAESPGLITICLLGYLLSAECTVFLDHENANKILNRPKRYNSGKLEEFVQGNLERECMEEKCSFEEAREVFENTERTTEFWKQYVDGDQCESNPCLNGGSCKDDINSYECWCPFGFEGKNCELDVTCNIKNGRCEQFCKNSADNKVVCSCTEGYRLAENQKSCEPAVPFPCGRVSVSQTSKLTRAETVFPDVDYVNSTEAETILDNITQSTQSFNDFTRVVGGEDAKPGQFPWQVVLNGKVDAFCGGSIVNEKWIVTAAHCVETGVKITVVAGEHNIEETEHTEQKRNVIRIIPHHNYNAAINKYNHDIALLELDEPLVLNSYVTPICIADKEYTNIFLKFGSGYVSGWGRVFHKGRSALVLQYLRVPLVDRATCLRSTKFTIYNNMFCAGFHEGGRDSCQGDSGGPHVTEVEGTSFLTGIISWGEECAMKGKYGIYTKVSRYVNWIKEKTKLTDKTHTCPPCPAPELLGGPSVFLFPPKPKDTLMISRTPEVTCVVVDVSHEDPEVKFNWYVDGVEVHNAKTKPREEQYNSTYRVVSVLTVLHQDWLNGKEYKCKVSNKALPAPIEKTISKAKGQPREPQVYTLPPSRDELTKNQVSLTCLVKGFYPSDIAVEWESNGQPENNYKTTPPVLDSDGSFFLYSKLTVDKSRWQQGNVFSCSVMHEALHNHYTQKSLSLSPGK

SEQ ID NO: 3 - DNA, 741 bp, Artificial Sequence
  Fc cassette from pSYN-FIX-030
atggagacagacacactcctgctatgggtactgctgctctgggttccaggttccactggtgacaaaactcacacatgcccaccgtgcccagcacctgaactcctgggaggaccgtcagtcttcctcttccccccaaaacccaaggacaccctcatgatctcccggacccctgaggtcacatgcgtggtggtggacgtgagccacgaagaccctgaggtcaagttcaactggtacgtggacggcgtggaggtgcataatgccaagacaaagccgcgggaggagcagtacaacagcacgtaccgtgtggtcagcgtcctcaccgtcctgcaccaggactggctgaatggcaaggagtacaagtgcaaggtctccaacaaagccctcccagcccccatcgagaaaaccatctccaaagccaaagggcagccccgagaaccacaggtgtacaccctgcccccatcccgcgatgagctgaccaagaaccaggtcagcctgacctgcctggtcaaaggcttctatcccagcgacatcgccgtggagtgggagagcaatgggcagccggagaacaactacaagaccacgcctcccgtgttggactccgacggctccttcttcctctacagcaagctcaccgtggacaagagcaggtggcagcaggggaacgtcttctcatgctccgtgatgcatgaggctctgcacaaccactacacgcagaagagcctctccctgtctccgggtaaa

SEQ ID NO: 4 - protein, 247 aa, Artificial Sequence
  Fc cassette from pSYN-FIX-030
  SIGNAL (-20)..(-1)
  mat_peptide (1)..(227)
METDTLLLWVLLLWVPGSTGDKTHTCPPCPAPELLGGPSVFLFPPKPKDTLMISRTPEVTCVVVDVSHEDPEVKFNWYVDGVEVHNAKTKPREEQYNSTYRVVSVLTVLHQDWLNGKEYKCKVSNKALPAPIEKTISKAKGQPREPQVYTLPPSRDELTKNQVSLTCLVKGFYPSDIAVEWESNGQPENNYKTTPPVLDSDGSFFLYSKLTVDKSRWQQGNVFSCSVMHEALHNHYTQKSLSLSPGK

SEQ ID NO: 5 - DNA, 5052 bp, Artificial Sequence
  B-Domain Deleted FVIIIFc
atgcaaatagagctctccacctgcttctttctgtgccttttgcgattctgctttagtgccaccagaagatactacctgggtgcagtggaactgtcatgggactatatgcaaagtgatctcggtgagctgcctgtggacgcaagatttcctcctagagtgccaaaatcttttccattcaacacctcagtcgtgtacaaaaagactctgtttgtagaattcacggatcaccttttcaacatcgctaagccaaggccaccctggatgggtctgctaggtcctaccatccaggctgaggtttatgatacagtggtcattacacttaagaacatggcttcccatcctgtcagtcttcatgctgttggtgtatcctactggaaagcttctgagggagctgaatatgatgatcagaccagtcaaagggagaaagaagatgataaagtcttccctggtggaagccatacatatgtctggcaggtcctgaaagagaatggtccaatggcctctgacccactgtgccttacctactcatatctttctcatgtggacctggtaaaagacttgaattcaggcctcattggagccctactagtatgtagagaagggagtctggccaaggaaaagacacagaccttgcacaaatttatactactttttgctgtatttgatgaagggaaaagttggcactcagaaacaaagaactccttgatgcaggatagggatgctgcatctgctcgggcctggcctaaaatgcacacagtcaatggttatgtaaacaggtctctgccaggtctgattggatgccacaggaaatcagtctattggcatgtgattggaatgggcaccactcctgaagtgcactcaatattcctcgaaggtcacacatttcttgtgaggaaccatcgccaggcgtccttggaaatctcgccaataactttccttactgctcaaacactcttgatggaccttggacagtttctactgttttgtcatatctcttcccaccaacatgatggcatggaagcttatgtcaaagtagacagctgtccagaggaaccccaactacgaatgaaaaataatgaagaagcggaagactatgatgatgatcttactgattctgaaatggatgtggtcaggtttgatgatgacaactctccttcctttatccaaattcgctcagttgccaagaagcatcctaaaacttgggtacattacattgctgctgaagaggaggactgggactatgctcccttagtcctcgcccccgatgacagaagttataaaagtcaatatttgaacaatggccctcagcggattggtaggaagtacaaaaaagtccgatttatggcatacacagatgaaacctttaagactcgtgaagctattcagcatgaatcaggaatcttgggacctttactttatggggaagttggagacacactgttgattatatttaagaatcaagcaagcagaccatataacatctaccctcacggaatcactgatgtccgtcctttgtattcaaggagattaccaaaaggtgtaaaacatttgaaggattttccaattctgccaggagaaatattcaaatataaatggacagtgactgtagaagatgggccaactaaatcagatcctcggtgcctgacccgctattactctagtttcgttaatatggagagagatctagcttcaggactcattggccctctcctcatctgctacaaagaatctgtagatcaaagaggaaaccagataatgtcagacaagaggaatgtcatcctgttttctgtatttgatgagaaccgaagctggtacctcacagagaatatacaacgctttctccccaatccagctggagtgcagcttgaggatccagagttccaagcctccaacatcatgcacagcatcaatggctatgtttttgatagtttgcagttgtcagtttgtttgcatgaggtggcatactggtacattctaagcattggagcacagactgacttcctttctgtcttcttctctggatataccttcaaacacaaaatggtctatgaagacacactcaccctattcccattctcaggagaaactgtcttcatgtcgatggaaaacccaggtctatggattctggggtgccacaactcagactttcggaacagaggcatgaccgccttactgaaggtttctagttgtgacaagaacactggtgattattacgaggacagttatgaagatatttcagcatacttgctgagtaaaaacaatgccattgaaccaagaagcttctctcaaaacccaccagtcttgaaacgccatcaacgggaaataactcgtactactcttcagtcagatcaagaggaaattgactatgatgataccatatcagttgaaatgaagaaggaagattttgacatttatgatgaggatgaaaatcagagcccccgcagctttcaaaagaaaacacgacactattttattgctgcagtggagaggctctgggattatgggatgagtagctccccacatgttctaagaaacagggctcagagtggcagtgtccctcagttcaagaaagttgttttccaggaatttactgatggctcctttactcagcccttataccgtggagaactaaatgaacatttgggactcctggggccatatataagagcagaagttgaagataatatcatggtaactttcagaaatcaggcctctcgtccctattccttctattctagccttatttcttatgaggaagatcagaggcaaggagcagaacctagaaaaaactttgtcaagcctaatgaaaccaaaacttacttttggaaagtgcaacatcatatggcacccactaaagatgagtttgactgcaaagcctgggcttatttctctgatgttgacctggaaaaagatgtgcactcaggcctgattggaccccttctggtctgccacactaacacactgaaccctgctcatgggagacaagtgacagtacaggaatttgctctgtttttcaccatctttgatgagaccaaaagctggtacttcactgaaaatatggaaagaaactgcagggctccctgcaatatccagatggaagatcccacttttaaagagaattatcgcttccatgcaatcaatggctacataatggatacactacctggcttagtaatggctcaggatcaaaggattcgatggtatctgctcagcatgggcagcaatgaaaacatccattctattcatttcagtggacatgtgttcactgtacgaaaaaaagaggagtataaaatggcactgtacaatctctatccaggtgtttttgagacagtggaaatgttaccatccaaagctggaatttggcgggtggaatgccttattggcgagcatctacatgctgggatgagcacactttttctggtgtacagcaataagtgtcagactcccctgggaatggcttctggacacattagagattttcagattacagcttcaggacaatatggacagtgggccccaaagctggccagacttcattattccggatcaatcaatgcctggagcaccaaggagcccttttcttggatcaaggtggatctgttggcaccaatgattattcacggcatcaagacccagggtgcccgtcagaagttctccagcctctacatctctcagtttatcatcatgtatagtcttgatgggaagaagtggcagacttatcgaggaaattccactggaaccttaatggtcttctttggcaatgtggattcatctgggataaaacacaatatttttaaccctccaattattgctcgatacatccgtttgcacccaactcattatagcattcgcagcactcttcgcatggagttgatgggctgtgatttaaatagttgcagcatgccattgggaatggagagtaaagcaatatcagatgcacagattactgcttcatcctactttaccaatatgtttgccacctggtctccttcaaaagctcgacttcacctccaagggaggagtaatgcctggagacctcaggtgaataatccaaaagagtggctgcaagtggacttccagaagacaatgaaagtcacaggagtaactactcagggagtaaaatctctgcttaccagcatgtatgtgaaggagttcctcatctccagcagtcaagatggccatcagtggactctcttttttcagaatggcaaagtaaaggtttttcagggaaatcaagactccttcacacctgtggtgaactctctagacccaccgttactgactcgctaccttcgaattcacccccagagttgggtgcaccagattgccctgaggatggaggttctgggctgcgaggcacaggacctctacgacaaaactcacacatgcccaccgtgcccagctccagaactcctgggcggaccgtcagtcttcctcttccccccaaaacccaaggacaccctcatgatctcccggacccctgaggtcacatgcgtggtggtggacgtgagccacgaagaccctgaggtcaagttcaactggtacgtggacggcgtggaggtgcataatgccaagacaaagccgcgggaggagcagtacaacagcacgtaccgtgtggtcagcgtcctcaccgtcctgcaccaggactggctgaatggcaaggagtacaagtgcaaggtctccaacaaagccctcccagcccccatcgagaaaaccatctccaaagccaaagggcagccccgagaaccacaggtgtacaccctgcccccatcccgggatgagctgaccaagaaccaggtcagcctgacctgcctggtcaaaggcttctatcccagcgacatcgccgtggagtgggagagcaatgggcagccggagaacaactacaagaccacgcctcccgtgttggactccgacggctccttcttcctctacagcaagctcaccgtggacaagagcaggtggcagcaggggaacgtcttctcatgctccgtgatgcatgaggctctgcacaaccactacacgcagaagagcctctccctgtctccgggtaaa

SEQ ID NO: 6 - protein, 1684 aa, Artificial Sequence
  B-Domain Deleted FVIIIFc
  SIGNAL (-19)..(-1)
  mat_peptide (1)..(1665)
MQIELSTCFFLCLLRFCFSATRRYYLGAVELSWDYMQSDLGELPVDARFPPRVPKSFPFNTSVVYKKTLFVEFTDHLFNIAKPRPPWMGLLGPTIQAEVYDTVVITLKNMASHPVSLHAVGVSYWKASEGAEYDDQTSQREKEDDKVFPGGSHTYVWQVLKENGPMASDPLCLTYSYLSHVDLVKDLNSGLIGALLVCREGSLAKEKTQTLHKFILLFAVFDEGKSWHSETKNSLMQDRDAASARAWPKMHTVNGYVNRSLPGLIGCHRKSVYWHVIGMGTTPEVHSIFLEGHTFLVRNHRQASLEISPITFLTAQTLLMDLGQFLLFCHISSHQHDGMEAYVKVDSCPEEPQLRMKNNEEAEDYDDDLTDSEMDVVRFDDDNSPSFIQIRSVAKKHPKTWVHYIAAEEEDWDYAPLVLAPDDRSYKSQYLNNGPQRIGRKYKKVRFMAYTDETFKTREAIQHESGILGPLLYGEVGDTLLIIFKNQASRPYNIYPHGITDVRPLYSRRLPKGVKHLKDFPILPGEIFKYKWTVTVEDGPTKSDPRCLTRYYSSFVNMERDLASGLIGPLLICYKESVDQRGNQIMSDKRNVILFSVFDENRSWYLTENIQRFLPNPAGVQLEDPEFQASNIMHSINGYVFDSLQLSVCLHEVAYWYILSIGAQTDFLSVFFSGYTFKHKMVYEDTLTLFPFSGETVFMSMENPGLWILGCHNSDFRNRGMTALLKVSSCDKNTGDYYEDSYEDISAYLLSKNNAIEPRSFSQNPPVLKRHQREITRTTLQSDQEEIDYDDTISVEMKKEDFDIYDEDENQSPRSFQKKTRHYFIAAVERLWDYGMSSSPHVLRNRAQSGSVPQFKKVVFQEFTDGSFTQPLYRGELNEHLGLLGPYIRAEVEDNIMVTFRNQASRPYSFYSSLISYEEDQRQGAEPRKNFVKPNETKTYFWKVQHHMAPTKDEFDCKAWAYFSDVDLEKDVHSGLIGPLLVCHTNTLNPAHGRQVTVQEFALFFTIFDETKSWYFTENMERNCRAPCNIQMEDPTFKENYRFHAINGYIMDTLPGLVMAQDQRIRWYLLSMGSNENIHSIHFSGHVFTVRKKEEYKMALYNLYPGVFETVEMLPSKAGIWRVECLIGEHLHAGMSTLFLVYSNKCQTPLGMASGHIRDFQITASGQYGQWAPKLARLHYSGSINAWSTKEPFSWIKVDLLAPMIIHGIKTQGARQKFSSLYISQFIIMYSLDGKKWQTYRGNSTGTLMVFFGNVDSSGIKHNIFNPPIIARYIRLHPTHYSIRSTLRMELMGCDLNSCSMPLGMESKAISDAQITASSYFTNMFATWSPSKARLHLQGRSNAWRPQVNNPKEWLQVDFQKTMKVTGVTTQGVKSLLTSMYVKEFLISSSQDGHQWTLFFQNGKVKVFQGNQDSFTPVVNSLDPPLLTRYLRIHPQSWVHQIALRMEVLGCEAQDLYDKTHTCPPCPAPELLGGPSVFLFPPKPKDTLMISRTPEVTCVVVDVSHEDPEVKFNWYVDGVEVHNAKTKPREEQYNSTYRVVSVLTVLHQDWLNGKEYKCKVSNKALPAPIEKTISKAKGQPREPQVYTLPPSRDELTKNQVSLTCLVKGFYPSDIAVEWESNGQPENNYKTTPPVLDSDGSFFLYSKLTVDKSRWQQGNVFSCSVMHEALHNHYTQKSLSLSPGK

SEQ ID NO: 7 - DNA, 741 bp, Artificial Sequence; identical to SEQ ID NO: 3
  Fc Sequence

SEQ ID NO: 8 - protein, 247 aa, Artificial Sequence; identical to SEQ ID NO: 4
  Fc chain
  SIGNAL (-20)..(-1)
  mat_peptide (-1)..(227)

SEQ ID NO: 9 - DNA, 7734 bp, Artificial Sequence
  Full Length FVIIIFc
atgcaaatagagctctccacctgcttctttctgtgccttttgcgattctgctttagtgccaccagaagatactacctgggtgcagtggaactgtcatgggactatatgcaaagtgatctcggtgagctgcctgtggacgcaagatttcctcctagagtgccaaaatcttttccattcaacacctcagtcgtgtacaaaaagactctgtttgtagaattcacggatcaccttttcaacatcgctaagccaaggccaccctggatgggtctgctaggtcctaccatccaggctgaggtttatgatacagtggtcattacacttaagaacatggcttcccatcctgtcagtcttcatgctgttggtgtatcctactggaaagcttctgagggagctgaatatgatgatcagaccagtcaaagggagaaagaagatgataaagtcttccctggtggaagccatacatatgtctggcaggtcctgaaagagaatggtccaatggcctctgacccactgtgccttacctactcatatctttctcatgtggacctggtaaaagacttgaattcaggcctcattggagccctactagtatgtagagaagggagtctggccaaggaaaagacacagaccttgcacaaatttatactactttttgctgtatttgatgaagggaaaagttggcactcagaaacaaagaactccttgatgcaggatagggatgctgcatctgctcgggcctggcctaaaatgcacacagtcaatggttatgtaaacaggtctctgccaggtctgattggatgccacaggaaatcagtctattggcatgtgattggaatgggcaccactcctgaagtgcactcaatattcctcgaaggtcacacatttcttgtgaggaaccatcgccaggcgtccttggaaatctcgccaataactttccttactgctcaaacactcttgatggaccttggacagtttctactgttttgtcatatctcttcccaccaacatgatggcatggaagcttatgtcaaagtagacagctgtccagaggaaccccaactacgaatgaaaaataatgaagaagcggaagactatgatgatgatcttactgattctgaaatggatgtggtcaggtttgatgatgacaactctccttcctttatccaaattcgctcagttgccaagaagcatcctaaaacttgggtacattacattgctgctgaagaggaggactgggactatgctcccttagtcctcgcccccgatgacagaagttataaaagtcaatatttgaacaatggccctcagcggattggtaggaagtacaaaaaagtccgatttatggcatacacagatgaaacctttaagactcgtgaagctattcagcatgaatcaggaatcttgggacctttactttatggggaagttggagacacactgttgattatatttaagaatcaagcaagcagaccatataacatctaccctcacggaatcactgatgtccgtcctttgtattcaaggagattaccaaaaggtgtaaaacatttgaaggattttccaattctgccaggagaaatattcaaatataaatggacagtgactgtagaagatgggccaactaaatcagatcctcggtgcctgacccgctattactctagtttcgttaatatggagagagatctagcttcaggactcattggccctctcctcatctgctacaaagaatctgtagatcaaagaggaaaccagataatgtcagacaagaggaatgtcatcctgttttctgtatttgatgagaaccgaagctggtacctcacagagaatatacaacgctttctccccaatccagctggagtgcagcttgaggatccagagttccaagcctccaacatcatgcacagcatcaatggctatgtttttgatagtttgcagttgtcagtttgtttgcatgaggtggcatactggtacattctaagcattggagcacagactgacttcctttctgtcttcttctctggatataccttcaaacacaaaatggtctatgaagacacactcaccctattcccattctcaggagaaactgtcttcatgtcgatggaaaacccaggtctatggattctggggtgccacaactcagactttcggaacagaggcatgaccgccttactgaaggtttctagttgtgacaagaacactggtgattattacgaggacagttatgaagatatttcagcatacttgctgagtaaaaacaatgccattgaaccaagaagcttctcccagaattcaagacaccctagcactaggcaaaagcaatttaatgccaccacaattccagaaaatgacatagagaagactgacccttggtttgcacacagaacacctatgcctaaaatacaaaatgtctcctctagtgatttgttgatgctcttgcgacagagtcctactccacatgggctatccttatctgatctccaagaagccaaatatgagactttttctgatgatccatcacctggagcaatagacagtaataacagcctgtctgaaatgacacacttcaggccacagctccatcacagtggggacatggtatttacccctgagtcaggcctccaattaagattaaatgagaaactggggacaactgcagcaacagagttgaagaaacttgatttcaaagtttctagtacatcaaataatctgatttcaacaattccatcagacaatttggcagcaggtactgataatacaagttccttaggacccccaagtatgccagttcattatgatagtcaattagataccactctatttggcaaaaagtcatctccccttactgagtctggtggacctctgagcttgagtgaagaaaataatgattcaaagttgttagaatcaggtttaatgaatagccaagaaagttcatggggaaaaaatgtatcgtcaacagagagtggtaggttatttaaagggaaaagagctcatggacctgctttgttgactaaagataatgccttattcaaagttagcatctctttgttaaagacaaacaaaacttccaataattcagcaactaatagaaagactcacattgatggcccatcattattaattgagaatagtccatcagtctggcaaaatatattagaaagtgacactgagtttaaaaaagtgacacctttgattcatgacagaatgcttatggacaaaaatgctacagctttgaggctaaatcatatgtcaaataaaactacttcatcaaaaaacatggaaatggtccaacagaaaaaagagggccccattccaccagatgcacaaaatccagatatgtcgttctttaagatgctattcttgccagaatcagcaaggtggatacaaaggactcatggaaagaactctctgaactctgggcaaggccccagtccaaagcaattagtatccttaggaccagaaaaatctgtggaaggtcagaatttcttgtctgagaaaaacaaagtggtagtaggaaagggtgaatttacaaaggacgtaggactcaaagagatggtttttccaagcagcagaaacctatttcttactaacttggataatttacatgaaaataatacacacaatcaagaaaaaaaaattcaggaagaaatagaaaagaaggaaacattaatccaagagaatgtagttttgcctcagatacatacagtgactggcactaagaatttcatgaagaaccttttcttactgagcactaggcaaaatgtagaaggttcatatgacggggcatatgctccagtacttcaagattttaggtcattaaatgattcaacaaatagaacaaagaaacacacagctcatttctcaaaaaaaggggaggaagaaaacttggaaggcttgggaaatcaaaccaagcaaattgtagagaaatatgcatgcaccacaaggatatctcctaatacaagccagcagaattttgtcacgcaacgtagtaagagagctttgaaacaattcagactcccactagaagaaacagaacttgaaaaaaggataattgtggatgacacctcaacccagtggtccaaaaacatgaaacatttgaccccgagcaccctcacacagatagactacaatgagaaggagaaaggggccattactcagtctcccttatcagattgccttacgaggagtcatagcatccctcaagcaaatagatctccattacccattgcaaaggtatcatcatttccatctattagacctatatatctgaccagggtcctattccaagacaactcttctcatcttccagcagcatcttatagaaagaaagattctggggtccaagaaagcagtcatttcttacaaggagccaaaaaaaataacctttctttagccattctaaccttggagatgactggtgatcaaagagaggttggctccctggggacaagtgccacaaattcagtcacatacaagaaagttgagaacactgttctcccgaaaccagacttgcccaaaacatctggcaaagttgaattgcttccaaaagttcacatttatcagaaggacctattccctacggaaactagcaatgggtctcctggccatctggatctcgtggaagggagccttcttcagggaacagagggagcgattaagtggaatgaagcaaacagacctggaaaagttccctttctgagagtagcaacagaaagctctgcaaagactccctccaagctattggatcctcttgcttgggataaccactatggtactcagataccaaaagaagagtggaaatcccaagagaagtcaccagaaaaaacagcttttaagaaaaaggataccattttgtccctgaacgcttgtgaaagcaatcatgcaatagcagcaataaatgagggacaaaataagcccgaaatagaagtcacctgggcaaagcaaggtaggactgaaaggctgtgctctcaaaacccaccagtcttgaaacgccatcaacgggaaataactcgtactactcttcagtcagatcaagaggaaattgactatgatgataccatatcagttgaaatgaagaaggaagattttgacatttatgatgaggatgaaaatcagagcccccgcagctttcaaaagaaaacacgacactattttattgctgcagtggagaggctctgggattatgggatgagtagctccccacatgttctaagaaacagggctcagagtggcagtgtccctcagttcaagaaagttgttttccaggaatttactgatggctcctttactcagcccttataccgtggagaactaaatgaacatttgggactcctggggccatatataagagcagaagttgaagataatatcatggtaactttcagaaatcaggcctctcgtccctattccttctattctagccttatttcttatgaggaagatcagaggcaaggagcagaacctagaaaaaactttgtcaagcctaatgaaaccaaaacttacttttggaaagtgcaacatcatatggcacccactaaagatgagtttgactgcaaagcctgggcttatttctctgatgttgacctggaaaaagatgtgcactcaggcctgattggaccccttctggtctgccacactaacacactgaaccctgctcatgggagacaagtgacagtacaggaatttgctctgtttttcaccatctttgatgagaccaaaagctggtacttcactgaaaatatggaaagaaactgcagggctccctgcaatatccagatggaagatcccacttttaaagagaattatcgcttccatgcaatcaatggctacataatggatacactacctggcttagtaatggctcaggatcaaaggattcgatggtatctgctcagcatgggcagcaatgaaaacatccattctattcatttcagtggacatgtgttcactgtacgaaaaaaagaggagtataaaatggcactgtacaatctctatccaggtgtttttgagacagtggaaatgttaccatccaaagctggaatttggcgggtggaatgccttattggcgagcatctacatgctgggatgagcacactttttctggtgtacagcaataagtgtcagactcccctgggaatggcttctggacacattagagattttcagattacagcttcaggacaatatggacagtgggccccaaagctggccagacttcattattccggatcaatcaatgcctggagcaccaaggagcccttttcttggatcaaggtggatctgttggcaccaatgattattcacggcatcaagacccagggtgcccgtcagaagttctccagcctctacatctctcagtttatcatcatgtatagtcttgatgggaagaagtggcagacttatcgaggaaattccactggaaccttaatggtcttctttggcaatgtggattcatctgggataaaacacaatatttttaaccctccaattattgctcgatacatccgtttgcacccaactcattatagcattcgcagcactcttcgcatggagttgatgggctgtgatttaaatagttgcagcatgccattgggaatggagagtaaagcaatatcagatgcacagattactgcttcatcctactttaccaatatgtttgccacctggtctccttcaaaagctcgacttcacctccaagggaggagtaatgcctggagacctcaggtgaataatccaaaagagtggctgcaagtggacttccagaagacaatgaaagtcacaggagtaactactcagggagtaaaatctctgcttaccagcatgtatgtgaaggagttcctcatctccagcagtcaagatggccatcagtggactctcttttttcagaatggcaaagtaaaggtttttcagggaaatcaagactccttcacacctgtggtgaactctctagacccaccgttactgactcgctaccttcgaattcacccccagagttgggtgcaccagattgccctgaggatggaggttctgggctgcgaggcacaggacctctacgacaaaactcacacatgcccaccgtgcccagctccagaactcctgggcggaccgtcagtcttcctcttccccccaaaacccaaggacaccctcatgatctcccggacccctgaggtcacatgcgtggtggtggacgtgagccacgaagaccctgaggtcaagttcaactggtacgtggacggcgtggaggtgcataatgccaagacaaagccgcgggaggagcagtacaacagcacgtaccgtgtggtcagcgtcctcaccgtcctgcaccaggactggctgaatggcaaggagtacaagtgcaaggtctccaacaaagccctcccagcccccatcgagaaaaccatctccaaagccaaagggcagccccgagaaccacaggtgtacaccctgcccccatcccgggatgagctgaccaagaaccaggtcagcctgacctgcctggtcaaaggcttctatcccagcgacatcgccgtggagtgggagagcaatgggcagccggagaacaactacaagaccacgcctcccgtgttggactccgacggctccttcttcctctacagcaagctcaccgtggacaagagcaggtggcagcaggggaacgtcttctcatgctccgtgatgcatgaggctctgcacaaccactacacgcagaagagcctctccctgtctccgggtaaa

SEQ ID NO: 10 - protein, 2578 aa, Artificial Sequence
  Full Length FVIIIFc
  SIGNAL (-19)..(-1)
  mat_peptide (1)..(2559)
MQIELSTCFFLCLLRFCFSATRRYYLGAVELSWDYMQSDLGELPVDARFPPRVPKSFPFNTSVVYKKTLFVEFTDHLFNIAKPRPPWMGLLGPTIQAEVYDTVVITLKNMASHPVSLHAVGVSYWKASEGAEYDDQTSQREKEDDKVFPGGSHTYVWQVLKENGPMASDPLCLTYSYLSHVDLVKDLNSGLIGALLVCREGSLAKEKTQTLHKFILLFAVFDEGKSWHSETKNSLMQDRDAASARAWPKMHTVNGYVNRSLPGLIGCHRKSVYWHVIGMGTTPEVHSIFLEGHTFLVRNHRQASLEISPITFLTAQTLLMDLGQFLLFCHISSHQHDGMEAYVKVDSCPEEPQLRMKNNEEAEDYDDDLTDSEMDVVRFDDDNSPSFIQIRSVAKKHPKTWVHYIAAEEEDWDYAPLVLAPDDRSYKSQYLNNGPQRIGRKYKKVRFMAYTDETFKTREAIQHESGILGPLLYGEVGDTLLIIFKNQASRPYNIYPHGITDVRPLYSRRLPKGVKHLKDFPILPGEIFKYKWTVTVEDGPTKSDPRCLTRYYSSFVNMERDLASGLIGPLLICYKESVDQRGNQIMSDKRNVILFSVFDENRSWYLTENIQRFLPNPAGVQLEDPEFQASNIMHSINGYVFDSLQLSVCLHEVAYWYILSIGAQTDFLSVFFSGYTFKHKMVYEDTLTLFPFSGETVFMSMENPGLWILGCHNSDFRNRGMTALLKVSSCDKNTGDYYEDSYEDISAYLLSKNNAIEPRSFSQNSRHPSTRQKQFNATTIPENDIEKTDPWFAHRTPMPKIQNVSSSDLLMLLRQSPTPHGLSLSDLQEAKYETFSDDPSPGAIDSNNSLSEMTHFRPQLHHSGDMVFTPESGLQLRLNEKLGTTAATELKKLDFKVSSTSNNLISTIPSDNLAAGTDNTSSLGPPSMPVHYDSQLDTTLFGKKSSPLTESGGPLSLSEENNDSKLLESGLMNSQESSWGKNVSSTESGRLFKGKRAHGPALLTKDNALFKVSISLLKTNKTSNNSATNRKTHIDGPSLLIENSPSVWQNILESDTEFKKVTPLIHDRMLMDKNATALRLNHMSNKTTSSKNMEMVQQKKEGPIPPDAQNPDMSFFKMLFLPESARWIQRTHGKNSLNSGQGPSPKQLVSLGPEKSVEGQNFLSEKNKVVVGKGEFTKDVGLKEMVFPSSRNLFLTNLDNLHENNTHNQEKKIQEEIEKKETLIQENVVLPQIHTVTGTKNFMKNLFLLSTRQNVEGSYDGAYAPVLQDFRSLNDSTNRTKKHTAHFSKKGEEENLEGLGNQTKQIVEKYACTTRISPNTSQQNFVTQRSKRALKQFRLPLEETELEKRIIVDDTSTQWSKNMKHLTPSTLTQIDYNEKEKGAITQSPLSDCLTRSHSIPQANRSPLPIAKVSSFPSIRPIYLTRVLFQDNSSHLPAASYRKKDSGVQESSHFLQGAKKNNLSLAILTLEMTGDQREVGSLGTSATNSVTYKKVENTVLPKPDLPKTSGKVELLPKVHIYQKDLFPTETSNGSPGHLDLVEGSLLQGTEGAIKWNEANRPGKVPFLRVATESSAKTPSKLLDPLAWDNHYGTQIPKEEWKSQEKSPEKTAFKKKDTILSLNACESNHAIAAINEGQNKPEIEVTWAKQGRTERLCSQNPPVLKRHQREITRTTLQSDQEEIDYDDTISVEMKKEDFDIYDEDENQSPRSFQKKTRHYFIAAVERLWDYGMSSSPHVLRNRAQSGSVPQFKKVVFQEFTDGSFTQPLYRGELNEHLGLLGPYIRAEVEDNIMVTFRNQASRPYSFYSSLISYEEDQRQGAEPRKNFVKPNETKTYFWKVQHHMAPTKDEFDCKAWAYFSDVDLEKDVHSGLIGPLLVCHTNTLNPAHGRQVTVQEFALFFTIFDETKSWYFTENMERNCRAPCNIQMEDPTFKENYRFHAINGYIMDTLPGLVMAQDQRIRWYLLSMGSNENIHSIHFSGHVFTVRKKEEYKMALYNLYPGVFETVEMLPSKAGIWRVECLIGEHLHAGMSTLFLVYSNKCQTPLGMASGHIRDFQITASGQYGQWAPKLARLHYSGSINAWSTKEPFSWIKVDLLAPMIIHGIKTQGARQKFSSLYISQFIIMYSLDGKKWQTYRGNSTGTLMVFFGNVDSSGIKHNIFNPPIIARYIRLHPTHYSIRSTLRMELMGCDLNSCSMPLGMESKAISDAQITASSYFTNMFATWSPSKARLHLQGRSNAWRPQVNNPKEWLQVDFQKTMKVTGVTTQGVKSLLTSMYVKEFLISSSQDGHQWTLFFQNGKVKVFQGNQDSFTPVVNSLDPPLLTRYLRIHPQSWVHQIALRMEVLGCEAQDLYDKTHTCPPCPAPELLGGPSVFLFPPKPKDTLMISRTPEVTCVVVDVSHEDPEVKFNWYVDGVEVHNAKTKPREEQYNSTYRVVSVLTVLHQDWLNGKEYKCKVSNKALPAPIEKTISKAKGQPREPQVYTLPPSRDELTKNQVSLTCLVKGFYPSDIAVEWESNGQPENNYKTTPPVLDSDGSFFLYSKLTVDKSRWQQGNVFSCSVMHEALHNHYTQKSLSLSPGK

SEQ ID NO: 11 - protein, 21 aa, Artificial Sequence
  Partial  B domain
SFSQNSRHPSQNPPVLKRHQR

SEQ ID NO: 12 - protein, 11 aa, Artificial Sequence
  albumin-binding peptide
DICLPRWGCLW

SEQ ID NO: 13 - protein, 32 aa, Artificial Sequence
  CTP peptide
DPRFQDSSSSKAPPPSLPSPSRLPGPSDTPIL

SEQ ID NO: 14 - protein, 28 aa, Artificial Sequence
  CTP peptide
SSSSKAPPPSLPSPSRLPGPSDTPILPQ

SEQ ID NO: 15 - protein, 20 aa, Artificial Sequence
  PAS peptide
ASPAAPAPASPAAPAPSAPA

SEQ ID NO: 16 - protein, 20 aa, Artificial Sequence
  PAS peptide
AAPASPAPAAPSAPAPAAPS

SEQ ID NO: 17 - protein, 20 aa, Artificial Sequence
  PAS peptide
APSSPSPSAPSSPSPASPSS

SEQ ID NO: 18 - protein, 19 aa, Artificial Sequence
  PAS peptide
APSSPSPSAPSSPSPASPS

SEQ ID NO: 19 - protein, 20 aa, Artificial Sequence
  PAS peptide
SSPSAPSPSSPASPSPSSPA

SEQ ID NO: 20 - protein, 24 aa, Artificial Sequence
  PAS peptide
AASPAAPSAPPAAASPAAPSAPPA

SEQ ID NO: 21 - protein, 20 aa, Artificial Sequence
  PAS peptide
ASAAAPAAASAAASAPSAAA